European Patent Application EP 4 389 894 A2, published June 26, 2024. Title: RIBOSWITCH MODULATED GENE THERAPY FOR RETINAL DISEASES. Applicant: The Medical College of Wisconsin, Inc. The sequence listing filed with the application follows.

SEQUENCE LISTING (80 sequences)

SEQ ID NO: 1 - DNA, 215 bp, synthetic construct
  misc_feature 1..215: note = synthetic
  source 1..215: mol_type = other DNA
cgtatcagcaggtcccataagctttcgacaattaacgagtgtgtactcgttctatcatctcacagttaaagtcgggagaataggagccgcacgggtcctgataccagcgtgagcggagagaatcttctttctgtctattagtgaagccacagatgtaatagacagaaagaagattctctccgcctacgcccttggcagcaccgtacggttcgatc

SEQ ID NO: 2 - DNA, 121 bp, synthetic construct
  misc_feature 1..121: note = synthetic
  source 1..121: mol_type = other DNA
ctagcgagagaatcttctttctgtctataaaagagagaatcttctttctgtctataaaagagagaatcttctttctgtctataaaagagagaatcttctttctgtctatgtcgaccctgca

SEQ ID NO: 3 - DNA, 286 bp, synthetic construct
  misc_feature 1..286: note = synthetic
  source 1..286: mol_type = other DNA
ggttggccactccctctctgcgcgctcgctcgctcactgaggccgggcgaccaaaggtcgcccgacgcccgggctttgcccgggcggcctcagtgagcgagcgagcgcgcagagagggagtggccaactccatcactaggggtacccctagtgatggagttggccactccctctctgcgcgctcgctcgctcactgaggccgcccgggcaaagcccgggcgtcgggcgacctttggtcgcccggcctcagtgagcgagcgagcgcgcagagagggagtggccaacc

SEQ ID NO: 4 - DNA, 236 bp, synthetic construct
  misc_feature 1..236: note = synthetic
  source 1..236: mol_type = other DNA
tcgactagagctcgctgatcagcctcgactgtgccttctagttgccagccatctgttgtttgcccctcccccgtgccttccttgaccctggaaggtgccactcccactgtcctttcctaataaaatgaggaaattgcatcgcattgtctgagtaggtgtcattctattctggggggtggggtggggcaggacagcaagggggaggattgggaagacaatagcaggcatgctgggga

SEQ ID NO: 5 - DNA, 202 bp, synthetic construct
  misc_feature 1..202: note = synthetic
  source 1..202: mol_type = other DNA
ggtgagcgggcgggacggcccttctcctccgggctgtaattagcgcttggtttaatgacggcttgtttcttttctgtggctgcgtgaaagccttgaggggctccgggagctagagcctctgctaaccatgttcatgccttcttctttttcctacagctcctgggcaacgtgctggttattgtgctgtctcatcattttggca

SEQ ID NO: 6 - DNA, 255 bp, synthetic construct
  misc_feature 1..255: note = synthetic
  source 1..255: mol_type = other DNA
catggtcgaggtgagccccacgttctgcttcactctccccatctcccccccctccccacccccaattttgtatttatttattttttaattattttgtgcagcgatgggggcggggggggggggggggcgcgcgccaggcggggcggggcggggcgaggggcggggcggggcgaggcggagaggtgcggcggcagccaatcagagcggcgcgctccgaaagtttccttttatggcgaggcggcggcggcggcggcc

SEQ ID NO: 7 - DNA, 255 bp, synthetic construct
  misc_feature 1..255: note = synthetic
  source 1..255: mol_type = other DNA
aattcggtacccctagttattaatagtaatcaattacggggtcattagttcatagcccatatatggagttccgcgttacataacttacggtaaatggcccgcctggctgaccgcccaacgacccccgcccattgacgtcaataatgacgtatgttcccatagtaacgccaatagggactttccattgacgtcaatgggtggactatttacggtaaactgcccacttggcagtacatcaagtgtatcatatgccaa

SEQ ID NO: 8 - DNA, 1374 bp, synthetic construct
  misc_feature 1..1374: note = synthetic
  source 1..1374: mol_type = other DNA
atggtatcatattgggacacaggagtcctcctgtgcgcccttttgagctgtcttttgctgacgggttcttcttcaggttctgataccgggagaccattcgttgaaatgtatagtgagatacccgaaattatacatatgactgaagggcgcgagctcgtcataccctgtcgggtaacaagtccaaacataacagtgaccctgaagaagttccctttggatactctcattcccgacgggaagcgaataatttgggactcaaggaagggatttatcatatctaatgcaacatataaggaaatagggctcctcacatgcgaagccacagtcaacgggcacctctacaaaactaattacctgacccatcgacagacaaataccatcattgatgtggttctgagtccatctcatggaatagagttgagtgtaggggagaagcttgttctcaattgcacagctagaaccgagttgaacgtgggtatcgattttaactgggaatacccatctagtaagcaccaacacaaaaaacttgtcaatcgagatttgaaaactcaatctggtagcgagatgaaaaagttcctgtcaactcttacaatcgatggcgtgacccggagtgatcaaggattgtatacctgcgccgccagctctggcctgatgactaaaaagaacagcacctttgtacgagtgcatgaaaaggataagactcatacatgccctccttgtcccgctccagagctgctgggaggtcccagtgttttcctcttcccaccaaagcccaaagatactctgatgattagccggacccctgaggtgacttgcgtcgtggtggatgtttcacatgaagatccagaagtgaagttcaattggtacgttgatggtgtggaggtacacaatgccaagactaaacctcgggaggaacagtataacagcacttacagagttgtcagcgtactcacagtgcttcatcaggactggttgaatggtaaggagtataagtgcaaagtgagtaataaggctctgccagcacccatagagaagacaatctcaaaggccaaaggccagccccgagaaccacaagtatacacactgccacctagtagagacgagttgacaaaaaatcaggtcagcctcacctgtctcgtgaaaggcttctaccctagcgacattgccgtagaatgggaaagcaacgggcaaccagaaaacaattataagacaacacctcccgttctcgatagtgacggaagtttcttcctgtatagcaaacttaccgtggataaatcaagatggcagcaaggtaatgtgtttagctgttcagtaatgcacgaagctctgcataaccactacacccaaaaatctttgtctctgtctccagggtga

SEQ ID NO: 9 - DNA, 3325 bp, synthetic construct
  misc_feature 1..3325: note = synthetic
  source 1..3325: mol_type = other DNA
ggttggccactccctctctgcgcgctcgctcgctcactgaggccgggcgaccaaaggtcgcccgacgcccgggctttgcccgggcggcctcagtgagcgagcgagcgcgcagagagggagtggccaactccatcactaggggttcctagatctgaattcggtacccctagttattaatagtaatcaattacggggtcattagttcatagcccatatatggagttccgcgttacataacttacggtaaatggcccgcctggctgaccgcccaacgacccccgcccattgacgtcaataatgacgtatgttcccatagtaacgccaatagggactttccattgacgtcaatgggtggactatttacggtaaactgcccacttggcagtacatcaagtgtatcatatgccaagtacgccccctattgacgtcaatgacggtaaatggcccgcctggcattatgcccagtacatgaccttatgggactttcctacttggcagtacatctacgtattagtcatcgctattaccatggtcgaggtgagccccacgttctgcttcactctccccatctcccccccctccccacccccaattttgtatttatttattttttaattattttgtgcagcgatgggggcggggggggggggggggcgcgcgccaggcggggcggggcggggcgaggggcggggcggggcgaggcggagaggtgcggcggcagccaatcagagcggcgcgctccgaaagtttccttttatggcgaggcggcggcggcggcggccctataaaaagcgaagcgcgcggcgggcgggagtcgctgcgacgctgccttcgccccgtgccccgctccgccgccgcctcgcgccgcccgccccggctctgactgaccgcgttactcccacaggtgagcgggcgggacggcccttctcctccgggctgtaattagcgcttggtttaatgacggcttgtttcttttctgtggctgcgtgaaagccttgaggggctccgggagctagagcctctgctaaccatgttcatgccttcttctttttcctacagctcctgggcaacgtgctggttattgtgctgtctcatcattttggcaaagaattcctcgaagatctaggcaacgcgtattgggatctcgaggcggccgcgccgccaccctagcgagagaatcttctttctgtctataaaagagagaatcttctttctgtctataaaagagagaatcttctttctgtctataaaagagagaatcttctttctgtctatgtcgaccctgcaatggtatcatattgggacacaggagtcctcctgtgcgcccttttgagctgtcttttgctgacgggttcttcttcaggttctgataccgggagaccattcgttgaaatgtatagtgagatacccgaaattatacatatgactgaagggcgcgagctcgtcataccctgtcgggtaacaagtccaaacataacagtgaccctgaagaagttccctttggatactctcattcccgacgggaagcgaataatttgggactcaaggaagggatttatcatatctaatgcaacatataaggaaatagggctcctcacatgcgaagccacagtcaacgggcacctctacaaaactaattacctgacccatcgacagacaaataccatcattgatgtggttctgagtccatctcatggaatagagttgagtgtaggggagaagcttgttctcaattgcacagctagaaccgagttgaacgtgggtatcgattttaactgggaatacccatctagtaagcaccaacacaaaaaacttgtcaatcgagatttgaaaactcaatctggtagcgagatgaaaaagttcctgtcaactcttacaatcgatggcgtgacccggagtgatcaaggattgtatacctgcgccgccagctctggcctgatgactaaaaagaacagcacctttgtacgagtgcatgaaaaggataagactcatacatgccctccttgtcccgctccagagctgctgggaggtcccagtgttttcctcttcccaccaaagcccaaagatactctgatgattagccggacccctgaggtgacttgcgtcgtggtggatgtttcacatgaagatccagaagtgaagttcaattggtacgttgatggtgtggaggtacacaatgccaagactaaacctcgggaggaacagtataacagcacttacagagttgtcagcgtactcacagtgcttcatcaggactggttgaatggtaaggagtataagtgcaaagtgagtaataaggctctgccagcacccatagagaagacaatctcaaaggccaaaggccagccccgagaaccacaagtatacacactgccacctagtagagacgagttgacaaaaaatcaggtcagcctcacctgtctcgtgaaaggcttctaccctagcgacattgccgtagaatgggaaagcaacgggcaaccagaaaacaattataagacaacacctcccgttctcgatagtgacggaagtttcttcctgtatagcaaacttaccgtggataaatcaagatggcagcaaggtaatgtgtttagctgttcagtaatgcacgaagctctgcataaccactacacccaaaaatctttgtctctgtctccagggtgagcgtatcagcaggtcccataagctttcgacaattaacgagtgtgtactcgttctatcatctcacagttaaagtcgggagaataggagccgcacgggtcctgataccagcgtgagcggagagaatcttctttctgtctattagtgaagccacagatgtaatagacagaaagaagattctctccgcctacgcccttggcagcaccgtacggttcgatcagcttattggtacatgataagtctcaggcatcgtacgatgtcgacctgcaggagtcggtcgactagagctcgctgatcagcctcgactgtgccttctagttgccagccatctgttgtttgcccctcccccgtgccttccttgaccctggaaggtgccactcccactgtcctttcctaataaaatgaggaaattgcatcgcattgtctgagtaggtgtcattctattctggggggtggggtggggcaggacagcaagggggaggattgggaagacaatagcaggcatgctggggagagatctaggaacccctagtgatggagttggccactccctctctgcgcgctcgctcgctcactgaggccgcccgggcaaagcccgggcgtcgggcgacctttggtcgcccggcctcagtgagcgagcgagcgcgcagagagggagtggccaacc

SEQ ID NO: 10 - DNA, 27 bp, synthetic construct
  misc_feature 1..27: note = synthetic
  source 1..27: mol_type = other DNA
gagagaatcttctttctgtctataaaa

SEQ ID NO: 11 - DNA, 168 bp, synthetic construct
  misc_feature 1..168: note = synthetic
  source 1..168: mol_type = other DNA
ctcgaggcgatcgcaaacaaacaaagctgtcaccggatgtgctttccggtctgatgagtccgttgtccaataccagcatcgtcttgatgcccttggcagtggatggggacggaggacgaaacagcaaaaagaaaaataaaaattttttttttaattaatcttgggccc

SEQ ID NO: 12 - DNA, 175 bp, synthetic construct
  misc_feature 1..175: note = synthetic
  source 1..175: mol_type = other DNA
ctcgaggcgatcgcaaacaaacaaagctgtcaccggatgtgctttccggtctgatgagtccgttgtccaaaacataccagatttcgatctggagaggtgaagaattcgaccacctggacgaggacggaggacgaaacagcaaaaagaaaaataaaaattaattaatcttgggccc

SEQ ID NO: 13 - DNA, 139 bp, synthetic construct
  misc_feature 1..139: note = synthetic
  source 1..139: mol_type = other DNA
atggccggcatggtcccagcctcctcgctggcgccggctgggcaaccacataccagccgaaaggcccttggcaggtgggcgaatgggacgcacaaatctctctagcttcccagagagaagcgagagaaaagtggctctc

SEQ ID NO: 14 - DNA, 135 bp, synthetic construct
  misc_feature 1..135: note = synthetic
  source 1..135: mol_type = other DNA
atggccggcatggtcccagcctcctcgctggcgccggctgggcaatgctataatcgcgtggatatggcacgcaagtttctaccgggcaccgtaaatgtccgactagtagcgaatgggacgcacaaatctctctag

SEQ ID NO: 15 - DNA, 134 bp, synthetic construct
  misc_feature 1..134: note = synthetic
  source 1..134: mol_type = other DNA
caaacaaacaaaggcgcgtcctggattcgtggtaaaacataccagatttcgatctggagaggtgaagaatacgaccacctgtagtatccagctgatgagtcccaaataggacgaaacgcgctaaacaaacaaac

SEQ ID NO: 16 - DNA, 123 bp, synthetic construct
  misc_feature 1..123: note = synthetic
  source 1..123: mol_type = other DNA
ctgaggtgcaggtacatccagctgacgagtcccaaataggacgaaagggagaggtgaagaatacgaccacctaggctcgaaagagcctaaaacatacctttcctggattccactgctatccac

SEQ ID NO: 17 - DNA, 286 bp, synthetic construct
  misc_feature 1..286: note = synthetic
  source 1..286: mol_type = other DNA
ctagcacgggtccctaaaacataccgtgagcgcgaaagcgcccccattttgagttagtgaagccacagatgtaactcaaaatgggggcgctttcccgcctacggagaggtgaagaatacgaccacctagaagcttattggtacatgataacaccccaaaatcgaagcacttcaaaaacaccccaaaatcgaagcacttcaaaaacaccccaaaatcgaagcacttcaaaaacaccccaaaatcgaagcacttcagtctcaggcatcgtacgatgtcgacctgcagg

SEQ ID NO: 18 - DNA, 1376 bp, synthetic construct
  misc_feature 1..1376: note = synthetic
  source 1..1376: mol_type = other DNA
aatgtccatgttgttctacactctgatcacagcttttctgatcggcatacaggcggaaccacactcagtctgataccgggagaccattcgttgaaatgtatagtgagatacccgaaattatacatatgactgaagggcgcgagctcgtcataccctgtcgggtaacaagtccaaacataacagtgaccctgaagaagttccctttggatactctcattcccgacgggaagcgaataatttgggactcaaggaagggatttatcatatctaatgcaacatataaggaaatagggctcctcacatgcgaagccacagtcaacgggcacctctacaaaactaattacctgacccatcgacagacaaataccatcattgatgtggttctgagtccatctcatggaatagagttgagtgtaggggagaagcttgttctcaattgcacagctagaaccgagttgaacgtgggtatcgattttaactgggaatacccatctagtaagcaccaacacaaaaaacttgtcaatcgagatttgaaaactcaatctggtagcgagatgaaaaagttcctgtcaactcttacaatcgatggcgtgacccggagtgatcaaggattgtatacctgcgccgccagctctggcctgatgactaaaaagaacagcacctttgtacgagtgcatgaaaaggataagactcatacatgccctccttgtcccgctccagagctgctgggaggtcccagtgttttcctcttcccaccaaagcccaaagatactctgatgattagccggacccctgaggtgacttgcgtcgtggtggatgtttcacatgaagatccagaagtgaagttcaattggtacgttgatggtgtggaggtacacaatgccaagactaaacctcgggaggaacagtataacagcacttacagagttgtcagcgtactcacagtgcttcatcaggactggttgaatggtaaggagtataagtgcaaagtgagtaataaggctctgccagcacccatagagaagacaatctcaaaggccaaaggccagccccgagaaccacaagtatacacactgccacctagtagagacgagttgacaaaaaatcaggtcagcctcacctgtctcgtgaaaggcttctaccctagcgacattgccgtagaatgggaaagcaacgggcaaccagaaaacaattataagacaacacctcccgttctcgatagtgacggaagtttcttcctgtatagcaaacttaccgtggataaatcaagatggcagcaaggtaatgtgtttagctgttcagtaatgcacgaagctctgcataaccactacacccaaaaatctttgtctctgtctccagggtgaaaacaaacaaaa

SEQ ID NO: 19 - DNA, 2960 bp, synthetic construct
  misc_feature 1..2960: note = synthetic
  source 1..2960: mol_type = other DNA
ggttggccactccctctctgcgcgctcgctcgctcactgaggccgggcgaccaaaggtcgcccgacgcccgggctttgcccgggcggcctcagtgagcgagcgagcgcgcagagagggagtggccaactccatcactaggggttcctagatctgaattcggtacccctagttattaatagtaatcaattacggggtcattagttcatagcccatatatggagttccgcgttacataacttacggtaaatggcccgcctggctgaccgcccaacgacccccgcccattgacgtcaataatgacgtatgttcccatagtaacgccaatagggactttccattgacgtcaatgggtggactatttacggtaaactgcccacttggcagtacatcaagtgtatcatatgccaagtacgccccctattgacgtcaatgacggtaaatggcccgcctggcattatgcccagtacatgaccttatgggactttcctacttggcagtacatctacgtattagtcatcgctattaccatggtcgaggtgagccccacgttctgcttcactctccccatctcccccccctccccacccccaattttgtatttatttattttttaattattttgtgcagcgatgggggcggggggggggggggggcgcgcgccaggcggggcggggcggggcgaggggcggggcggggcgaggcggagaggtgcggcggcagccaatcagagcggcgcgctccgaaagtttccttttatggcgaggcggcggcggcggcggccctataaaaagcgaagcgcgcggcgggcgggagtcgctgcgacgctgccttcgccccgtgccccgctccgccgccgcctcgcgccgcccgccccggctctgactgaccgcgttactcccacaggtgagcgggcgggacggcccttctcctccgggctgtaattagcgcttggtttaatgacggcttgtttcttttctgtggctgcgtgaaagccttgaggggctccgggagctagagcctctgctaaccatgttcatgccttcttctttttcctacagctcctgggcaacgtgctggttattgtgctgtctcatcattttggcaaagaattcctcgaagatctaggcaacgcgtctcgaggcggccgccgccaccaatggtatcatattgggacacaggagtcctcctgtgcgcccttttgagctgtcttttgctgacgggttcttcttcaggttctgataccgggagaccattcgttgaaatgtatagtgagatacccgaaattatacatatgactgaagggcgcgagctcgtcataccctgtcgggtaacaagtccaaacataacagtgaccctgaagaagttccctttggatactctcattcccgacgggaagcgaataatttgggactcaaggaagggatttatcatatctaatgcaacatataaggaaatagggctcctcacatgcgaagccacagtcaacgggcacctctacaaaactaattacctgacccatcgacagacaaataccatcattgatgtggttctgagtccatctcatggaatagagttgagtgtaggggagaagcttgttctcaattgcacagctagaaccgagttgaacgtgggtatcgattttaactgggaatacccatctagtaagcaccaacacaaaaaacttgtcaatcgagatttgaaaactcaatctggtagcgagatgaaaaagttcctgtcaactcttacaatcgatggcgtgacccggagtgatcaaggattgtatacctgcgccgccagctctggcctgatgactaaaaagaacagcacctttgtacgagtgcatgaaaaggataagactcatacatgccctccttgtcccgctccagagctgctgggaggtcccagtgttttcctcttcccaccaaagcccaaagatactctgatgattagccggacccctgaggtgacttgcgtcgtggtggatgtttcacatgaagatccagaagtgaagttcaattggtacgttgatggtgtggaggtacacaatgccaagactaaacctcgggaggaacagtataacagcacttacagagttgtcagcgtactcacagtgcttcatcaggactggttgaatggtaaggagtataagtgcaaagtgagtaataaggctctgccagcacccatagagaagacaatctcaaaggccaaaggccagccccgagaaccacaagtatacacactgccacctagtagagacgagttgacaaaaaatcaggtcagcctcacctgtctcgtgaaaggcttctaccctagcgacattgccgtagaatgggaaagcaacgggcaaccagaaaacaattataagacaacacctcccgttctcgatagtgacggaagtttcttcctgtatagcaaacttaccgtggataaatcaagatggcagcaaggtaatgtgtttagctgttcagtaatgcacgaagctctgcataaccactacacccaaaaatctttgtctctgtctccagggtgagcggccgcatcggctagcaaagcttcctgcaggagtcggtcgactagagctcgctgatcagcctcgactgtgccttctagttgccagccatctgttgtttgcccctcccccgtgccttccttgaccctggaaggtgccactcccactgtcctttcctaataaaatgaggaaattgcatcgcattgtctgagtaggtgtcattctattctggggggtggggtggggcaggacagcaagggggaggattgggaagacaatagcaggcatgctggggagagatctaggaacccctagtgatggagttggccactccctctctgcgcgctcgctcgctcactgaggccgcccgggcaaagcccgggcgtcgggcgacctttggtcgcccggcctcagtgagcgagcgagcgcgcagagagggagtggccaacc

SEQ ID NO: 20 - DNA, 1374 bp, synthetic construct; identical to SEQ ID NO: 8
  misc_feature 1..1374: note = synthetic
  source 1..1374: mol_type = other DNA

SEQ ID NO: 21 - DNA, 153 bp, synthetic construct
  misc_feature 1..153: note = synthetic
  source 1..153: mol_type = other DNA
gaacgcctcctaacgtctggtcacgaccctgcgtgagcgaccccattgttcaggtttgtattcttttggccactgactgagaatacaaatgaacaatgggggcgcctacgcagcccctcgaaatcacgagggagacgagataagggggcgttt

SEQ ID NO: 22 - DNA, 155 bp, synthetic construct
  misc_feature 1..155: note = synthetic
  source 1..155: mol_type = other DNA
gaacgcctcctaacgtctggtcacgaccctgcgtgagcgaccctgagttccttccctaaatacttttggccactgactgagtatttaggaggaactcaggggggcgcctacgcagcccctcgaaatcacgagggagacgagataagggggcgttt

SEQ ID NO: 23 - DNA, 155 bp, synthetic construct
  misc_feature 1..155: note = synthetic
  source 1..155: mol_type = other DNA
gaacgcctcctaacgtctggtcacgaccctgcgtgagcgaccaagagttaacgtgtcgatctcttttggccactgactgagagatcgacgttaactcttgggggcgcctacgcagcccctcgaaatcacgagggagacgagataagggggcgttt

SEQ ID NO: 24 - DNA, 155 bp, synthetic construct
  misc_feature 1..155: note = synthetic
  source 1..155: mol_type = other DNA
gaacgcctcctaacgtctggtcacgaccctgcgtgagcgacccttccctaaatagtatagatcttttggccactgactgagatctatactttagggaaggggggcgcctacgcagcccctcgaaatcacgagggagacgagataagggggcgttt

SEQ ID NO: 25 - DNA, 155 bp, synthetic construct
  misc_feature 1..155: note = synthetic
  source 1..155: mol_type = other DNA
gaacgcctcctaacgtctggtcacgaccctgcgtgagcgaccgtgtcgatcttggctcaactcttttggccactgactgagcgtgtcgattggctcaactggggcgcctacgcagcccctcgaaatcacgagggagacgagataagggggcgttt

SEQ ID NO: 26 - DNA, 127 bp, synthetic construct
  misc_feature 1..127: note = synthetic
  source 1..127: mol_type = other DNA
gaacgcctccttgataccagctgcgtgagcgaccccattgttcaggtttgtattcttttggccactgactgagaatacaaatgaacaatgggggcgcctacgcgcccttggcagcaagggggcgttt

SEQ ID NO: 27 - DNA, 129 bp, synthetic construct
  misc_feature 1..129: note = synthetic
  source 1..129: mol_type = other DNA
gaacgcctccttgataccagctgcgtgagcgaccctgagttccttccctaaatacttttggccactgactgagtatttaggaggaactcaggggggcgcctacgcgcccttggcagcaagggggcgttt

SEQ ID NO: 28 - DNA, 129 bp, synthetic construct
  misc_feature 1..129: note = synthetic
  source 1..129: mol_type = other DNA
gaacgcctccttgataccagctgcgtgagcgaccaagagttaacgtgtcgatctcttttggccactgactgagagatcgacgttaactcttgggggcgcctacgcgcccttggcagcaagggggcgttt

SEQ ID NO: 29 - DNA, 129 bp, synthetic construct
  misc_feature 1..129: note = synthetic
  source 1..129: mol_type = other DNA
gaacgcctccttgataccagctgcgtgagcgacccttccctaaatagtatagatcttttggccactgactgagatctatactttagggaaggggggcgcctacgcgcccttggcagcaagggggcgttt

SEQ ID NO: 30 - DNA, 129 bp, synthetic construct
  misc_feature 1..129: note = synthetic
  source 1..129: mol_type = other DNA
gaacgcctccttgataccagctgcgtgagcgaccgtgtcgatcttggctcaactcttttggccactgactgagcgtgtcgattggctcaactggggcgcctacgcgcccttggcagcaagggggcgttt

SEQ ID NO: 31 - DNA, 151 bp, synthetic construct
  misc_feature 1..151: note = synthetic
  source 1..151: mol_type = other DNA
gaacgcctcctagaggtgaagaatacgaccaccttgcgtgagcgaccccattgttcaggtttgtattcttttggccactgactgagaatacaaatgaacaatgggggcgcctacgcaggctcgaaagagcctaaaacataagggggcgttt

SEQ ID NO: 32 - DNA, 153 bp, synthetic construct
  misc_feature 1..153: note = synthetic
  source 1..153: mol_type = other DNA
gaacgcctcctagaggtgaagaatacgaccaccttgcgtgagcgaccctgagttccttccctaaatacttttggccactgactgagtatttaggaggaactcaggggggcgcctacgcaggctcgaaagagcctaaaacataagggggcgttt

SEQ ID NO: 33 - DNA, 153 bp, synthetic construct
  misc_feature 1..153: note = synthetic
  source 1..153: mol_type = other DNA
gaacgcctcctagaggtgaagaatacgaccaccttgcgtgagcgaccaagagttaacgtgtcgatctcttttggccactgactgagagatcgacgttaactcttgggggcgcctacgcaggctcgaaagagcctaaaacataagggggcgttt

SEQ ID NO: 34 - DNA, 153 bp, synthetic construct
  misc_feature 1..153: note = synthetic
  source 1..153: mol_type = other DNA
gaacgcctcctagaggtgaagaatacgaccaccttgcgtgagcgacccttccctaaatagtatagatcttttggccactgactgagatctatactttagggaaggggggcgcctacgcaggctcgaaagagcctaaaacataagggggcgttt

SEQ ID NO: 35 - DNA, 153 bp, synthetic construct
  misc_feature 1..153: note = synthetic
  source 1..153: mol_type = other DNA
gaacgcctcctagaggtgaagaatacgaccaccttgcgtgagcgaccgtgtcgatcttggctcaactcttttggccactgactgagcgtgtcgattggctcaactggggcgcctacgcaggctcgaaagagcctaaaacataagggggcgttt

SEQ ID NO: 36 - DNA, 2077 bp, synthetic construct
  misc_feature 1..2077: note = synthetic
  source 1..2077: mol_type = other DNA
aatggtcagctactgggacaccggggtcctgctgtgcgcgctgctcagctgtctgcttctcacaggatctagttcaggttcaaaattaaaagatcctgaactgagtttaaaaggcacccagcacatcatgcaagcaggccagacactgcatctccaatgcaggggggaagcagcccataaatggtctttgcctgaaatggtgagtaaggaaagcgaaaggctgagcataactaaatctgcctgtggaagaaatggcaaacaattctgcagtactttaaccttgaacacagctcaagcaaaccacactggcttctacagctgcaaatatctagctgtacctacttcaaagaagaaggaaacagaatctgcaatctatatatttattagtgatacaggtagacctttcgtagagatgtacagtgaaatccccgaaattatacacatgactgaaggaagggagctcgtcattccctgccgggttacgtcacctaacatcactgttactttaaaaaagtttccacttgacactttgatccctgatggaaaacgcataatctgggacagtagaaagggcttcatcatatcaaatgcaacgtacaaagaaatagggcttctgacctgtgaagcaacagtcaatgggcatttgtataagacaaactatctcacacatcgacaaaccaatacaatcatagatgtccaaataagcacaccacgcccagtcaaattacttagaggccatactcttgtcctcaattgtactgctaccactcccttgaacacgagagttcaaatgacctggagttaccctgatgaaaaaaataagagagcttccgtaaggcgacgaattgaccaaagcaattcccatgccaacatattctacagtgttcttactattgacaaaatgcagaacaaagacaaaggactttatacttgtcgtgtaaggagtggaccatcattcaaatctgttaacacctcagtgcatatatatgataaagcattcatcactgtgaaacatcgaaaacagcaggtgcttgaaaccgtagctggcaagcggtcttaccggctctctatgaaagtgaaggcatttccctcgccggaagttgtatggttaaaagatgggttacctgcgactgagaaatctgctcgctatttgactcgtggctactcgttaattatcaaggacgtaactgaagaggatgcagggaattatacaatcttgctgagcataaaacagtcaaatgtgtttaaaaacctcactgccactctaattgtcaatgtgaaaccccagatttacgaaaaggccgtgtcatcgtttccagacccggctctctacccactgggcagcagacaaatcctgacttgtaccgcatatggtatccctcaacctacaatcaagtggttctggcacccctgtaaccataatcattccgaagcaaggtgtgacttttgttccaataatgaagagtcctttatcctggatgctgacagcaacatgggaaacagaattgagagcatcactcagcgcatggcaataatagaaggaaagaataagatggctagcaccttggttgtggctgactctagaatttctggaatctacatttgcatagcttccaataaagttgggactgtgggaagaaacataagcttttatatcacagatgtgccaaatgggtttcatgttaacttggaaaaaatgccgacggaaggagaggacctgaaactgtcttgcacagttaacaagttcttatacagagacgttacttggattttactgcggacagttaataacagaacaatgcactacagtattagcaagcaaaaaatggccatcactaaggagcactccatcactcttaatcttaccatcatgaatgtttccctgcaagattcaggcacctatgcctgcagagccaggaatgtatacacaggggaagaaatcctccagaagaaagaaattacaatcagaggtgagcactgcaacaaaaaggctgttttctctcggatctccaaatttaaaagcacaaggaatgattgtaccacacaaagtaatgtaaaacattaaaaacaaacaaaa

SEQ ID NO: 37 - DNA, 155 bp, synthetic construct
  misc_feature 1..155: note = synthetic
  source 1..155: mol_type = other DNA
gaacgcctcctaacgtctggtcacgaccctgcgtgagcgaccagacgaagagtgtcctagatcttttggccactgactgagatctaggactcttcgtctgggggcgcctacgcagcccctcgaaatcacgagggagacgagataagggggcgttt

SEQ ID NO: 38 - DNA, 155 bp, synthetic construct
  misc_feature 1..155: note = synthetic
  source 1..155: mol_type = other DNA
gaacgcctcctaacgtctggtcacgaccctgcgtgagcgaccgctttccgactcgtattgatcttttggccactgactgagatcaatacgtcggaaagcgggggcgcctacgcagcccctcgaaatcacgagggagacgagataagggggcgttt

SEQ ID NO: 39 - DNA, 155 bp, synthetic construct
  misc_feature 1..155: note = synthetic
  source 1..155: mol_type = other DNA
gaacgcctcctaacgtctggtcacgaccctgcgtgagcgaccaccttctttaccgtttgttacttttggccactgactgagtaacaaactaaagaaggtgggggcgcctacgcagcccctcgaaatcacgagggagacgagataagggggcgttt

SEQ ID NO: 40 - DNA, 155 bp, synthetic construct
  misc_feature 1..155: note = synthetic
  source 1..155: mol_type = other DNA
gaacgcctcctaacgtctggtcacgaccctgcgtgagcgacccgtttgttaagacgtcatgacttttggccactgactgagtcatgacgttaacaaacggggggcgcctacgcagcccctcgaaatcacgagggagacgagataagggggcgttt

SEQ ID NO: 41 - DNA, 155 bp, synthetic construct
  misc_feature 1..155: note = synthetic
  source 1..155: mol_type = other DNA
gaacgcctcctaacgtctggtcacgaccctgcgtgagcgacgcaaatatctagctgtacctacttttggccactgactgagtaggtacatagatatttgcggggcgcctacgcagcccctcgaaatcacgagggagacgagataagggggcgttt

SEQ ID NO: 42 - DNA, 129 bp, synthetic construct
  misc_feature 1..129: note = synthetic
  source 1..129: mol_type = other DNA
gaacgcctccttgataccagctgcgtgagcgaccagacgaagagtgtcctagatcttttggccactgactgagatctaggactcttcgtctgggggcgcctacgcgcccttggcagcaagggggcgttt

SEQ ID NO: 43 - DNA, 129 bp, synthetic construct
  misc_feature 1..129: note = synthetic
  source 1..129: mol_type = other DNA
gaacgcctccttgataccagctgcgtgagcgaccgctttccgactcgtattgatcttttggccactgactgagatcaatacgtcggaaagcgggggcgcctacgcgcccttggcagcaagggggcgttt

SEQ ID NO: 44 - DNA, 129 bp, synthetic construct
  misc_feature 1..129: note = synthetic
  source 1..129: mol_type = other DNA
gaacgcctccttgataccagctgcgtgagcgaccaccttctttaccgtttgttacttttggccactgactgagtaacaaactaaagaaggtgggggcgcctacgcgcccttggcagcaagggggcgttt

SEQ ID NO: 45 - DNA, 129 bp, synthetic construct
  misc_feature 1..129: note = synthetic
  source 1..129: mol_type = other DNA
gaacgcctccttgataccagctgcgtgagcgacccgtttgttaagacgtcatgacttttggccactgactgagtcatgacgttaacaaacggggggcgcctacgcgcccttggcagcaagggggcgttt

SEQ ID NO: 46 - DNA, 129 bp, synthetic construct
  misc_feature 1..129: note = synthetic
  source 1..129: mol_type = other DNA
gaacgcctccttgataccagctgcgtgagcgacgcaaatatctagctgtacctacttttggccactgactgagtaggtacatagatatttgcggggcgcctacgcgcccttggcagcaagggggcgttt

SEQ ID NO: 47 - DNA, 153 bp, synthetic construct
  misc_feature 1..153: note = synthetic
  source 1..153: mol_type = other DNA
gaacgcctcctagaggtgaagaatacgaccaccttgcgtgagcgaccagacgaagagtgtcctagatcttttggccactgactgagatctaggactcttcgtctgggggcgcctacgcaggctcgaaagagcctaaaacataagggggcgttt

SEQ ID NO: 48 - DNA, 153 bp, synthetic construct
  misc_feature 1..153: note = synthetic
  source 1..153: mol_type = other DNA
gaacgcctcctagaggtgaagaatacgaccaccttgcgtgagcgaccgctttccgactcgtattgatcttttggccactgactgagatcaatacgtcggaaagcgggggcgcctacgcaggctcgaaagagcctaaaacataagggggcgttt

SEQ ID NO: 49 - DNA, 153 bp, synthetic construct
  misc_feature 1..153: note = synthetic
  source 1..153: mol_type = other DNA
gaacgcctcctagaggtgaagaatacgaccaccttgcgtgagcgaccaccttctttaccgtttgttacttttggccactgactgagtaacaaactaaagaaggtgggggcgcctacgcaggctcgaaagagcctaaaacataagggggcgttt

SEQ ID NO: 50 - DNA, 153 bp, synthetic construct
  misc_feature 1..153: note = synthetic
  source 1..153: mol_type = other DNA
gaacgcctcctagaggtgaagaatacgaccaccttgcgtgagcgacccgtttgttaagacgtcatgacttttggccactgactgagtcatgacgttaacaaacggggggcgcctacgcaggctcgaaagagcctaaaacataagggggcgttt

SEQ ID NO: 51 - DNA, 142 bp, synthetic construct
  misc_feature 1..142: note = synthetic
  source 1..142: mol_type = other DNA
gaacgcctcctagaggtgaagaatacgaccaccttgcgtgagcgacgcaaatatctagctgtacctacttttggccactgactgagtaggtacatagatatttgcggggcgcctacgcaggctcgaaagagcctaaaacata

SEQ ID NO: 52 - DNA, 1815 bp, synthetic construct
  misc_feature 1..1815: note = synthetic
  source 1..1815: mol_type = other DNA
atgcttgcccgggccctgcttctgtgtgcggtattggcactgagtcacacagccaacccgtgctgctcacacccatgtcagaatcggggagtttgcatgtcagtagggtttgaccaatataagtgcgactgtacccggacaggcttttatggagaaaattgttctacacccgaatttttgacgaggattaagctctttctgaagcctacaccaaatacagtccattatatcctcacgcacttcaagggtttttggaatgtcgtaaacaacattccgtttctgagaaatgcgataatgtcttacgtccttacatcccggagccaccttattgactcacccccaacatacaacgccgactacggatacaaaagttgggaagctttctccaacctgtcttactacacgcgagcattgcctcctgtacccgacgattgcccgacgccgttgggggtgaaaggaaaaaagcagctcccggactcaaacgaaatagtagagaaattgttgcttcgccgaaaatttataccagacccgcagggtagcaatatgatgtttgcgttcttcgctcagcacttcactcaccaattctttaagacagaccacaagagaggtcccgcattcacgaatggccttggacacggcgtcgacttgaaccacatatatggggagacattggccagacaaaggaaacttcgattgtttaaggatgggaaaatgaaataccaaattattgatggcgagatgtatcctccaacagtgaaggatacgcaagcggagatgatttatccaccgcaggtaccagagcatttgcggttcgcggtggggcaggaagtatttggacttgttcccggtctgatgatgtacgccacaatatggctccgggagcataatcgcgtgtgtgacgtacttaagcaagagcacccggaatggggcgacgagcaactttttcaaacgagtcgactgattctcattggggaaacgattaaaatagtgatcgaagattatgtgcaacatctttctggttaccactttaagttgaagttcgatcctgagctgcttttcaataaacaattccagtatcaaaacagaatcgccgcggagttcaacacgctgtatcattggcatcccctgttgcccgatacttttcaaatccatgaccagaaatacaattaccagcaatttatatataataactctatcctcctggagcatggcattacacaattcgttgaaagtttcacaaggcagatcgcaggaagagttgcgggtggccggaatgtgccgcctgccgtgcaaaaggtatcacaggctagcatcgaccaatcaaggcaaatgaagtaccagtcttttaatgagtacaggaaaaggttcatgctgaagccttacgagagctttgaagaactgacgggcgaaaaggaaatgtccgcggaactggaagcgttgtacggagatattgatgcggtagagctctaccccgcgcttctggtcgaaaagccccggccagatgccattttcggggaaaccatggttgaagtgggcgccccattcagtttgaaaggtctgatgggtaatgtaatttgcagtccggcgtactggaagccttccacttttggtggggaagtggggtttcaaattatcaatacggcctcaattcagtctctgatttgtaacaatgttaagggatgtccctttacatcttttagtgtaccggaccccgagcttattaagaccgtgaccataaatgcttcaagctctagaagtggtcttgatgatatcaaccccacagttttgcttaaggaaaggagcacggagctctaa

SEQ ID NO: 53 - DNA, 894 bp, synthetic construct
  misc_feature 1..894: note = synthetic
  source 1..894: mol_type = other DNA
atgagcatgaacaactcaaaacagttggtctccccagcagcggcccttttgtccaacacaacgtgtcagactgagaatagactcagtgtattttttagcgtgatttttatgaccgtcggtatcctgtctaactctcttgccatagcaatattgatgaaagcctatcagcgattccggcaaaagtctaaggcgtcatttttgttgttggcaagcgggcttgtcatcacggactttttcgggcacctcattaacggagccatagccgtgttcgtttatgcttcagacaaagagtggatacgattcgatcagagcaatgtgctttgcagtatctttggcatatgtatggtgtttagtggattgtgtccactcttgcttgggagcgtgatggctattgaaagatgcatcggggtgactaaacctatctttcacagtaccaaaattacatctaagcacgtcaagatgatgttgtccggggtgtgtctttttgctgtctttattgcgttgttgccaatactgggccacagggactacaaaattcaggcctcacgcacttggtgcttctataacactgaggatattaaagactgggaggataggttttatcttcttcttttctcattcctcggtctgctcgcactgggggtatcccttttgtgtaacgctatcacaggtatcaccttgttgcgcgttaaatttaagagccaacagcatcgccaggggaggtcacatcacctcgaaatggtaatacagttgctcgcgatcatgtgtgttagttgtatctgctggtcacccttcttgggatatagaataattctgaatggaaaagaaaagtacaaagtctatgaagaacagagcgattttctgcatcgattgcaatggcccactttggaataa

SEQ ID NO: 54 - DNA, 2771 bp, synthetic construct
  misc_feature 1..2771: note = synthetic
  source 1..2771: mol_type = other DNA
aatgcttgcccgggccctgcttctgtgtgcggtattggcactgagtcacacagccaacccgtgctgctcacacccatgtcagaatcggggagtttgcatgtcagtagggtttgaccaatataagtgcgactgtacccggacaggcttttatggagaaaattgttctacacccgaatttttgacgaggattaagctctttctgaagcctacaccaaatacagtccattatatcctcacgcacttcaagggtttttggaatgtcgtaaacaacattccgtttctgagaaatgcgataatgtcttacgtccttacatcccggagccaccttattgactcacccccaacatacaacgccgactacggatacaaaagttgggaagctttctccaacctgtcttactacacgcgagcattgcctcctgtacccgacgattgcccgacgccgttgggggtgaaaggaaaaaagcagctcccggactcaaacgaaatagtagagaaattgttgcttcgccgaaaatttataccagacccgcagggtagcaatatgatgtttgcgttcttcgctcagcacttcactcaccaattctttaagacagaccacaagagaggtcccgcattcacgaatggccttggacacggcgtcgacttgaaccacatatatggggagacattggccagacaaaggaaacttcgattgtttaaggatgggaaaatgaaataccaaattattgatggcgagatgtatcctccaacagtgaaggatacgcaagcggagatgatttatccaccgcaggtaccagagcatttgcggttcgcggtggggcaggaagtatttggacttgttcccggtctgatgatgtacgccacaatatggctccgggagcataatcgcgtgtgtgacgtacttaagcaagagcacccggaatggggcgacgagcaactttttcaaacgagtcgactgattctcattggggaaacgattaaaatagtgatcgaagattatgtgcaacatctttctggttaccactttaagttgaagttcgatcctgagctgcttttcaataaacaattccagtatcaaaacagaatcgccgcggagttcaacacgctgtatcattggcatcccctgttgcccgatacttttcaaatccatgaccagaaatacaattaccagcaatttatatataataactctatcctcctggagcatggcattacacaattcgttgaaagtttcacaaggcagatcgcaggaagagttgcgggtggccggaatgtgccgcctgccgtgcaaaaggtatcacaggctagcatcgaccaatcaaggcaaatgaagtaccagtcttttaatgagtacaggaaaaggttcatgctgaagccttacgagagctttgaagaactgacgggcgaaaaggaaatgtccgcggaactggaagcgttgtacggagatattgatgcggtagagctctaccccgcgcttctggtcgaaaagccccggccagatgccattttcggggaaaccatggttgaagtgggcgccccattcagtttgaaaggtctgatgggtaatgtaatttgcagtccggcgtactggaagccttccacttttggtggggaagtggggtttcaaattatcaatacggcctcaattcagtctctgatttgtaacaatgttaagggatgtccctttacatcttttagtgtaccggaccccgagcttattaagaccgtgaccataaatgcttcaagctctagaagtggtcttgatgatatcaaccccacagttttgcttaaggaaaggagcacggagctcggaagcggagctactaacttcagcctgctgaagcaggctggagacgtcgaggagaaccctggacctagcatgaacaactcaaaacagttggtctccccagcagcggcccttttgtccaacacaacgtgtcagactgagaatagactcagtgtattttttagcgtgatttttatgaccgtcggtatcctgtctaactctcttgccatagcaatattgatgaaagcctatcagcgattccggcaaaagtctaaggcgtcatttttgttgttggcaagcgggcttgtcatcacggactttttcgggcacctcattaacggagccatagccgtgttcgtttatgcttcagacaaagagtggatacgattcgatcagagcaatgtgctttgcagtatctttggcatatgtatggtgtttagtggattgtgtccactcttgcttgggagcgtgatggctattgaaagatgcatcggggtgactaaacctatctttcacagtaccaaaattacatctaagcacgtcaagatgatgttgtccggggtgtgtctttttgctgtctttattgcgttgttgccaatactgggccacagggactacaaaattcaggcctcacgcacttggtgcttctataacactgaggatattaaagactgggaggataggttttatcttcttcttttctcattcctcggtctgctcgcactgggggtatcccttttgtgtaacgctatcacaggtatcaccttgttgcgcgttaaatttaagagccaacagcatcgccaggggaggtcacatcacctcgaaatggtaatacagttgctcgcgatcatgtgtgttagttgtatctgctggtcacccttcttgggatatagaataattctgaatggaaaagaaaagtacaaagtctatgaagaacagagcgattttctgcatcgattgcaatggcccactttggaataaa

SEQ ID NO: 55 - DNA, 1812 bp, synthetic construct
  misc_feature 1..1812: note = synthetic
  source 1..1812: mol_type = other DNA
atgcttgcccgggccctgcttctgtgtgcggtattggcactgagtcacacagccaacccgtgctgctcacacccatgtcagaatcggggagtttgcatgtcagtagggtttgaccaatataagtgcgactgtacccggacaggcttttatggagaaaattgttctacacccgaatttttgacgaggattaagctctttctgaagcctacaccaaatacagtccattatatcctcacgcacttcaagggtttttggaatgtcgtaaacaacattccgtttctgagaaatgcgataatgtcttacgtccttacatcccggagccaccttattgactcacccccaacatacaacgccgactacggatacaaaagttgggaagctttctccaacctgtcttactacacgcgagcattgcctcctgtacccgacgattgcccgacgccgttgggggtgaaaggaaaaaagcagctcccggactcaaacgaaatagtagagaaattgttgcttcgccgaaaatttataccagacccgcagggtagcaatatgatgtttgcgttcttcgctcagcacttcactcaccaattctttaagacagaccacaagagaggtcccgcattcacgaatggccttggacacggcgtcgacttgaaccacatatatggggagacattggccagacaaaggaaacttcgattgtttaaggatgggaaaatgaaataccaaattattgatggcgagatgtatcctccaacagtgaaggatacgcaagcggagatgatttatccaccgcaggtaccagagcatttgcggttcgcggtggggcaggaagtatttggacttgttcccggtctgatgatgtacgccacaatatggctccgggagcataatcgcgtgtgtgacgtacttaagcaagagcacccggaatggggcgacgagcaactttttcaaacgagtcgactgattctcattggggaaacgattaaaatagtgatcgaagattatgtgcaacatctttctggttaccactttaagttgaagttcgatcctgagctgcttttcaataaacaattccagtatcaaaacagaatcgccgcggagttcaacacgctgtatcattggcatcccctgttgcccgatacttttcaaatccatgaccagaaatacaattaccagcaatttatatataataactctatcctcctggagcatggcattacacaattcgttgaaagtttcacaaggcagatcgcaggaagagttgcgggtggccggaatgtgccgcctgccgtgcaaaaggtatcacaggctagcatcgaccaatcaaggcaaatgaagtaccagtcttttaatgagtacaggaaaaggttcatgctgaagccttacgagagctttgaagaactgacgggcgaaaaggaaatgtccgcggaactggaagcgttgtacggagatattgatgcggtagagctctaccccgcgcttctggtcgaaaagccccggccagatgccattttcggggaaaccatggttgaagtgggcgccccattcagtttgaaaggtctgatgggtaatgtaatttgcagtccggcgtactggaagccttccacttttggtggggaagtggggtttcaaattatcaatacggcctcaattcagtctctgatttgtaacaatgttaagggatgtccctttacatcttttagtgtaccggaccccgagcttattaagaccgtgaccataaatgcttcaagctctagaagtggtcttgatgatatcaaccccacagttttgcttaaggaaaggagcacggagctc

SEQ ID NO: 56 - DNA, 66 bp, synthetic construct
  misc_feature 1..66: note = synthetic
  source 1..66: mol_type = other DNA
ggaagcggagctactaacttcagcctgctgaagcaggctggagacgtcgaggagaaccctggacct

SEQ ID NO: 57 - DNA, 891 bp, synthetic construct
  misc_feature 1..891: note = synthetic
  source 1..891: mol_type = other DNA
agcatgaacaactcaaaacagttggtctccccagcagcggcccttttgtccaacacaacgtgtcagactgagaatagactcagtgtattttttagcgtgatttttatgaccgtcggtatcctgtctaactctcttgccatagcaatattgatgaaagcctatcagcgattccggcaaaagtctaaggcgtcatttttgttgttggcaagcgggcttgtcatcacggactttttcgggcacctcattaacggagccatagccgtgttcgtttatgcttcagacaaagagtggatacgattcgatcagagcaatgtgctttgcagtatctttggcatatgtatggtgtttagtggattgtgtccactcttgcttgggagcgtgatggctattgaaagatgcatcggggtgactaaacctatctttcacagtaccaaaattacatctaagcacgtcaagatgatgttgtccggggtgtgtctttttgctgtctttattgcgttgttgccaatactgggccacagggactacaaaattcaggcctcacgcacttggtgcttctataacactgaggatattaaagactgggaggataggttttatcttcttcttttctcattcctcggtctgctcgcactgggggtatcccttttgtgtaacgctatcacaggtatcaccttgttgcgcgttaaatttaagagccaacagcatcgccaggggaggtcacatcacctcgaaatggtaatacagttgctcgcgatcatgtgtgttagttgtatctgctggtcacccttcttgggatatagaataattctgaatggaaaagaaaagtacaaagtctatgaagaacagagcgattttctgcatcgattgcaatggcccactttggaataa

SEQ ID NO: 58 - DNA, 4621 bp, synthetic construct
  misc_feature 1..4621: note = synthetic
  source 1..4621: mol_type = other DNA
ggttggccactccctctctgcgcgctcgctcgctcactgaggccgggcgaccaaaggtcgcccgacgcccgggctttgcccgggcggcctcagtgagcgagcgagcgcgcagagagggagtggccaactccatcactaggggttcctagatctgaattcggtacccctagttattaatagtaatcaattacggggtcattagttcatagcccatatatggagttccgcgttacataacttacggtaaatggcccgcctggctgaccgcccaacgacccccgcccattgacgtcaataatgacgtatgttcccatagtaacgccaatagggactttccattgacgtcaatgggtggactatttacggtaaactgcccacttggcagtacatcaagtgtatcatatgccaagtacgccccctattgacgtcaatgacggtaaatggcccgcctggcattatgcccagtacatgaccttatgggactttcctacttggcagtacatctacgtattagtcatcgctattaccatggtcgaggtgagccccacgttctgcttcactctccccatctcccccccctccccacccccaattttgtatttatttattttttaattattttgtgcagcgatgggggcggggggggggggggggcgcgcgccaggcggggcggggcggggcgaggggcggggcggggcgaggcggagaggtgcggcggcagccaatcagagcggcgcgctccgaaagtttccttttatggcgaggcggcggcggcggcggccctataaaaagcgaagcgcgcggcgggcgggagtcgctgcgacgctgccttcgccccgtgccccgctccgccgccgcctcgcgccgcccgccccggctctgactgaccgcgttactcccacaggtgagcgggcgggacggcccttctcctccgggctgtaattagcgcttggtttaatgacggcttgtttcttttctgtggctgcgtgaaagccttgaggggctccgggagctagagcctctgctaaccatgttcatgccttcttctttttcctacagctcctgggcaacgtgctggttattgtgctgtctcatcattttggcaaagaattcctcgaagatctaggcaactcgagaaacaaacaaactgaggtgcaggtacatccagctgacgagtcccaaataggacgaaagggagaggtgaagaatacgaccacctaggctcgaaagagcctaaaacataccttcctggattccactgctatccacaaaaagaaaaataaaaagccaccatgcttgcccgggccctgcttctgtgtgcggtattggcactgagtcacacagccaacccgtgctgctcacacccatgtcagaatcggggagtttgcatgtcagtagggtttgaccaatataagtgcgactgtacccggacaggcttttatggagaaaattgttctacacccgaatttttgacgaggattaagctctttctgaagcctacaccaaatacagtccattatatcctcacgcacttcaagggtttttggaatgtcgtaaacaacattccgtttctgagaaatgcgataatgtcttacgtccttacatcccggagccaccttattgactcacccccaacatacaacgccgactacggatacaaaagttgggaagctttctccaacctgtcttactacacgcgagcattgcctcctgtacccgacgattgcccgacgccgttgggggtgaaaggaaaaaagcagctcccggactcaaacgaaatagtagagaaattgttgcttcgccgaaaatttataccagacccgcagggtagcaatatgatgtttgcgttcttcgctcagcacttcactcaccaattctttaagacagaccacaagagaggtcccgcattcacgaatggccttggacacggcgtcgacttgaaccacatatatggggagacattggccagacaaaggaaacttcgattgtttaaggatgggaaaatgaaataccaaattattgatggcgagatgtatcctccaacagtgaaggatacgcaagcggagatgatttatccaccgcaggtaccagagcatttgcggttcgcggtggggcaggaagtatttggacttgttcccggtctgatgatgtacgccacaatatggctccgggagcataatcgcgtgtgtgacgtacttaagcaagagcacccggaatggggcgacgagcaactttttcaaacgagtcgactgattctcattggggaaacgattaaaatagtgatcgaagattatgtgcaacatctttctggttaccactttaagttgaagttcgatcctgagctgcttttcaataaacaattccagtatcaaaacagaatcgccgcggagttcaacacgctgtatcattggcatcccctgttgcccgatacttttcaaatccatgaccagaaatacaattaccagcaatttatatataataactctatcctcctggagcatggcattacacaattcgttgaaagtttcacaaggcagatcgcaggaagagttgcgggtggccggaatgtgccgcctgccgtgcaaaaggtatcacaggctagcatcgaccaatcaaggcaaatgaagtaccagtcttttaatgagtacaggaaaaggttcatgctgaagccttacgagagctttgaagaactgacgggcgaaaaggaaatgtccgcggaactggaagcgttgtacggagatattgatgcggtagagctctaccccgcgcttctggtcgaaaagccccggccagatgccattttcggggaaaccatggttgaagtgggcgccccattcagtttgaaaggtctgatgggtaatgtaatttgcagtccggcgtactggaagccttccacttttggtggggaagtggggtttcaaattatcaatacggcctcaattcagtctctgatttgtaacaatgttaagggatgtccctttacatcttttagtgtaccggaccccgagcttattaagaccgtgaccataaatgcttcaagctctagaagtggtcttgatgatatcaaccccacagttttgcttaaggaaaggagcacggagctcggaagcggagctactaacttcagcctgctgaagcaggctggagacgtcgaggagaaccctggacctagcatgaacaactcaaaacagttggtctccccagcagcggcccttttgtccaacacaacgtgtcagactgagaatagactcagtgtattttttagcgtgatttttatgaccgtcggtatcctgtctaactctcttgccatagcaatattgatgaaagcctatcagcgattccggcaaaagtctaaggcgtcatttttgttgttggcaagcgggcttgtcatcacggactttttcgggcacctcattaacggagccatagccgtgttcgtttatgcttcagacaaagagtggatacgattcgatcagagcaatgtgctttgcagtatctttggcatatgtatggtgtttagtggattgtgtccactcttgcttgggagcgtgatggctattgaaagatgcatcggggtgactaaacctatctttcacagtaccaaaattacatctaagcacgtcaagatgatgttgtccggggtgtgtctttttgctgtctttattgcgttgttgccaatactgggccacagggactacaaaattcaggcctcacgcacttggtgcttctataacactgaggatattaaagactgggaggataggttttatcttcttcttttctcattcctcggtctgctcgcactgggggtatcccttttgtgtaacgctatcacaggtatcaccttgttgcgcgttaaatttaagagccaacagcatcgccaggggaggtcacatcacctcgaaatggtaatacagttgctcgcgatcatgtgtgttagttgtatctgctggtcacccttcttgggatatagaataattctgaatggaaaagaaaagtacaaagtctatgaagaacagagcgattttctgcatcgattgcaatggcccactttggaataaaaacaaacaaactgagatgcaggtacatcccactgatgagtcccaaataggacgaaagggagaggtgaagaatacgaccacctaggctcgaaagagcctaaaacataccttctgggattccactgctatccacaaaaagaaaaataaaaagcggccgctgcaggagtcggtcgactagagctcgctgatcagcctcgactgtgccttctagttgccagccatctgttgtttgcccctcccccgtgccttccttgaccctggaaggtgccactcccactgtcctttcctaataaaatgaggaaattgcatcgcattgtctgagtaggtgtcattctattctggggggtggggtggggcaggacagcaagggggaggattgggaagacaatagcaggcatgctggggagagatctaggaacccctagtgatggagttggccactccctctctgcgcgctcgctcgctcactgaggccgcccgggcaaagcccgggcgtcgggcgacctttggtcgcccggcctcagtgagcgagcgagcgcgcagagagggagtggccaacc

SEQ ID NO: 59 - DNA, 122 bp, synthetic construct
  misc_feature 1..122: note = synthetic
  source 1..122: mol_type = other DNA
ctgaggtgcaggtacatccagctgacgagtcccaaataggacgaaagggagaggtgaagaatacgaccacctaggctcgaaagagcctaaaacataccttcctggattccactgctatccac

SEQ ID NO: 60 - DNA, 1812 bp, synthetic construct; identical to SEQ ID NO: 55
  misc_feature 1..1812: note = synthetic
  source 1..1812: mol_type = other DNA

SEQ ID NO: 61 - DNA, 66 bp, synthetic construct; identical to SEQ ID NO: 56
  misc_feature 1..66: note = synthetic
  source 1..66: mol_type = other DNA

SEQ ID NO: 62 - DNA, 891 bp, synthetic construct; identical to SEQ ID NO: 57
  misc_feature 1..891: note = synthetic
  source 1..891: mol_type = other DNA

SEQ ID NO: 63 - DNA, 122 bp, synthetic construct
  misc_feature 1..122: note = synthetic
  source 1..122: mol_type = other DNA
ctgagatgcaggtacatcccactgatgagtcccaaataggacgaaagggagaggtgaagaatacgaccacctaggctcgaaagagcctaaaacataccttctgggattccactgctatccac

SEQ ID NO: 64 - DNA, 168 bp, synthetic construct; identical to SEQ ID NO: 11
  misc_feature 1..168: note = synthetic
  source 1..168: mol_type = other DNA

SEQ ID NO: 65 - DNA, 139 bp, synthetic construct; identical to SEQ ID NO: 13
  misc_feature 1..139: note = synthetic
  source 1..139: mol_type = other DNA

SEQ ID NO: 66 - DNA, 135 bp, synthetic construct; identical to SEQ ID NO: 14
  misc_feature 1..135: note = synthetic
  source 1..135: mol_type = other DNA

SEQ ID NO: 67 - DNA, 134 bp, synthetic construct; identical to SEQ ID NO: 15
  misc_feature 1..134: note = synthetic
  source 1..134: mol_type = other DNA

SEQ ID NO: 68 - DNA, 104 bp, synthetic construct
  misc_feature 1..104: note = synthetic
  source 1..104: mol_type = other DNA
gagagaatcttctttctgtctataaaagagagaatcttctttctgtctataaaagagagaatcttctttctgtctataaaagagagaatcttctttctgtctat

SEQ ID NO: 69 - DNA, 124 bp, synthetic construct
  misc_feature 1..124: note = synthetic
  source 1..124: mol_type = other DNA
gcggccgcgctagcacgggtcctgataccagcgtgagcggagagaatcttctttctgtctattagtgaagccacagatgtaatagacagaaagaagattctctccgcctacgcccttggcagca

SEQ ID NO: 70 - DNA, 21 bp, synthetic construct
  misc_feature 1..21: note = synthetic
  source 1..21: mol_type = other DNA
tatttagggaaggaactcagg

SEQ ID NO: 71 - DNA, 21 bp, synthetic construct
  misc_feature 1..21: note = synthetic
  source 1..21: mol_type = other DNA
aatacaaacctgaacaatggg

SEQ ID NO: 72 - DNA, 21 bp, synthetic construct
  misc_feature 1..21: note = synthetic
  source 1..21: mol_type = other DNA
agttgagccaagatcgacacg

SEQ ID NO: 73 - DNA, 21 bp, synthetic construct
  misc_feature 1..21: note = synthetic
  source 1..21: mol_type = other DNA
atctatactatttagggaagg

SEQ ID NO: 74 - DNA, 21 bp, synthetic construct
  misc_feature 1..21: note = synthetic
  source 1..21: mol_type = other DNA
agatcgacacgttaactcttg

SEQ ID NO: 75 - DNA, 21 bp, synthetic construct
  misc_feature 1..21: note = synthetic
  source 1..21: mol_type = other DNA
taggtacagctagatatttgc

SEQ ID NO: 76 - DNA, 21 bp, synthetic construct
  misc_feature 1..21: note = synthetic
  source 1..21: mol_type = other DNA
tcatgacgtcttaacaaacgg

SEQ ID NO: 77 - DNA, 21 bp, synthetic construct
  misc_feature 1..21: note = synthetic
  source 1..21: mol_type = other DNA
taacaaacggtaaagaaggtg

SEQ ID NO: 78 - DNA, 21 bp, synthetic construct
  misc_feature 1..21: note = synthetic
  source 1..21: mol_type = other DNA
atcaatacgagtcggaaagcg

SEQ ID NO: 79 - DNA, 21 bp, synthetic construct
  misc_feature 1..21: note = synthetic
  source 1..21: mol_type = other DNA
atctaggacactcttcgtctg

SEQ ID NO: 80 - RNA, 13 nt, synthetic construct
  misc_feature 1..13: note = Synthetic
  source 1..13: mol_type = other RNA
aaaaaaaaaaaaa